European Patent Specification EP 3 200 794 B1, published July 22, 2026. Title: A Compound for Anti-Cancer Therapy That Acts By Targeting GOF Mutant P53 and Stimulates P73 to Restore the P53 Pathway Signaling. Applicant: The Penn State Research Foundation El-Diery, Wafik S. Zhang, Shengliang. The sequence listing filed with the application follows.

SEQUENCE LISTING (10 sequences)

SEQ ID NO: 1 - DNA, 20 bp, Artificial sequence
  Chemically synthesized
gaggttggctctgactgtac

SEQ ID NO: 2 - DNA, 20 bp, Artificial sequence
  Chemically synthesized
tccgtcccagtagattacca

SEQ ID NO: 3 - DNA, 18 bp, Artificial sequence
  Chemically synthesized
tgtccgtcagaacccatg

SEQ ID NO: 4 - DNA, 20 bp, Artificial sequence
  Chemically synthesized
aaagtcgaagttccatcgct

SEQ ID NO: 5 - DNA, 20 bp, Artificial sequence
  Chemically synthesized
gacgacctcaacgcacagta

SEQ ID NO: 6 - DNA, 22 bp, Artificial sequence
  Chemically synthesized
aggagtcccatgatgagattgt

SEQ ID NO: 7 - DNA, 20 bp, Artificial sequence
  Chemically synthesized
gcagagctggaagtcgagtg

SEQ ID NO: 8 - DNA, 23 bp, Artificial sequence
  Chemically synthesized
gagcagaagagtttggatatcag

SEQ ID NO: 9 - DNA, 19 bp, Artificial sequence
  Chemically synthesized
ctgggctacactgagcacc

SEQ ID NO: 10 - DNA, 21 bp, Artificial sequence
  Chemically synthesized
aagtggtcgttgagggcaatg